European Patent Application EP 4 620 968 A1, published September 24, 2025. Title: Peptide Having Activity of Skin Whitening and Uses Thereof. Applicant: CAREGEN CO., LTD. The sequence listing filed with the application follows.

SEQUENCE LISTING (5 sequences)

SEQ ID NO: 1 - protein, 9 aa, synthetic construct
KQTPLVFKK

SEQ ID NO: 2 - DNA, 20 bp, synthetic construct
  source 1..20: mol_type = other DNA
tgctagcagcctctctctcc

SEQ ID NO: 3 - DNA, 20 bp, synthetic construct
  source 1..20: mol_type = other DNA
cttcaaggggaaccagatga

SEQ ID NO: 4 - DNA, 20 bp, synthetic construct
  source 1..20: mol_type = other DNA
ggagccaaaagggtcatcat

SEQ ID NO: 5 - DNA, 20 bp, synthetic construct
  source 1..20: mol_type = other DNA
gtgatggcatggactgtggt